European Patent Application EP 4 631 519 A1, published October 15, 2025. Title: METHOD FOR LOWERING BLOOD GLUCOSE LEVEL. Applicant: Baosheng Biomedical Research Co., Ltd. Application EP. The sequence listing filed with the application follows.

SEQUENCE LISTING (1 sequence)

SEQ ID NO: 1 - protein, 204 aa, Momordica charantia
MKNFALLCFLFALIASTEVRICKSDASPDAVLDIDGKKLRAGVNYYILPVIRGRGGGLTLGNIGHDKCPLHVVQEQFEISNGLPATFAPVNPKKGVVRVSTDLNVEFEASTVCAKSTVWKLDKFDESTRQWLVAIGGIRGNPGQETLDNWFKIEKHGKDYKFVFCPSVCKFCKVICKDVGIFIKNGNRALALSDTPFPVMFKKV